European Patent Specification EP 3 848 706 B1, published July 19, 2023. Title: Coupling Method. Applicant: Oxford Nanopore Technologies Limited. The sequence listing filed with the application follows.

SEQUENCE LISTING (41 sequences)

SEQ ID NO: 1 - DNA, 558 bp, Artificial sequence
  Mycobacterium smegmatis porin A mutant (D90N/D91N/D93N/D118R/D134R/E139K)
atgggtctggataatgaactgagcctggtggacggtcaagatcgtaccctgacggtgcaacaatgggatacctttctgaatggcgtttttccgctggatcgtaatcgcctgacccgtgaatggtttcattccggtcgcgcaaaatatatcgtcgcaggcccgggtgctgacgaattcgaaggcacgctggaactgggttatcagattggctttccgtggtcactgggcgttggtatcaacttctcgtacaccacgccgaatattctgatcaacaatggtaacattaccgcaccgccgtttggcctgaacagcgtgattacgccgaacctgtttccgggtgttagcatctctgcccgtctgggcaatggtccgggcattcaagaagtggcaacctttagtgtgcgcgtttccggcgctaaaggcggtgtcgcggtgtctaacgcccacggtaccgttacgggcgcggccggcggtgtcctgctgcgtccgttcgcgcgcctgattgcctctaccggcgacagcgttacgacctatggcgaaccgtggaatatgaactaa

SEQ ID NO: 2 - protein, 184 aa, Artificial sequence
  Mycobacterium smegmatis porin A mutant (D90N/D91N/D93N/D118R/D134R/E139K)
GLDNELSLVDGQDRTLTVQQWDTFLNGVFPLDRNRLTREWFHSGRAKYIVAGPGADEFEGTLELGYQIGFPWSLGVGINFSYTTPNILINNGNITAPPFGLNSVITPNLFPGVSISARLGNGPGIQEVATFSVRVSGAKGGVAVSNAHGTVTGAAGGVLLRPFARLIASTGDSVTTYGEPWNMN

SEQ ID NO: 3 - DNA, 882 bp, Artificial sequence
  alpha-hemolysin mutant (M111R)
atggcagattctgatattaatattaaaaccggtactacagatattggaagcaatactacagtaaaaacaggtgatttagtcacttatgataaagaaaatggcatgcacaaaaaagtattttatagttttatcgatgataaaaatcacaataaaaaactgctagttattagaacaaaaggtaccattgctggtcaatatagagtttatagcgaagaaggtgctaacaaaagtggtttagcctggccttcagcctttaaggtacagttgcaactacctgataatgaagtagctcaaatatctgattactatccaagaaattcgattgatacaaaagagtataggagtactttaacttatggattcaacggtaatgttactggtgatgatacaggaaaaattggcggccttattggtgcaaatgtttcgattggtcatacactgaaatatgttcaacctgatttcaaaacaattttagagagcccaactgataaaaaagtaggctggaaagtgatatttaacaatatggtgaatcaaaattggggaccatacgatcgagattcttggaacccggtatatggcaatcaacttttcatgaaaactagaaatggttctatgaaagcagcagataacttccttgatcctaacaaagcaagttctctattatcttcagggttttcaccagacttcgctacagttattactatggatagaaaagcatccaaacaacaaacaaatatagatgtaatatacgaacgagttcgtgatgattaccaattgcattggacttcaacaaattggaaaggtaccaatactaaagataaatggacagatcgttcttcagaaagatataaaatcgattgggaaaaagaagaaatgacaaat

SEQ ID NO: 4 - protein, 293 aa, Artificial sequence
  alpha-hemolysin mutant (M111R)
ADSDINIKTGTTDIGSNTTVKTGDLVTYDKENGMHKKVFYSFIDDKNHNKKLLVIRTKGTIAGQYRVYSEEGANKSGLAWPSAFKVQLQLPDNEVAQISDYYPRNSIDTKEYRSTLTYGFNGNVTGDDTGKIGGLIGANVSIGHTLKYVQPDFKTILESPTDKKVGWKVIFNNMVNQNWGPYDRDSWNPVYGNQLFMKTRNGSMKAADNFLDPNKASSLLSSGFSPDFATVITMDRKASKQQTNIDVIYERVRDDYQLHWTSTNWKGTNTKDKWTDRSSERYKIDWEKEEMTN

SEQ ID NO: 5 - DNA, 1830 bp, bacteriophage phi AR29
atgaaacacatgccgcgtaaaatgtatagctgcgcgtttgaaaccacgaccaaagtggaagattgtcgcgtttgggcctatggctacatgaacatcgaagatcattctgaatacaaaatcggtaacagtctggatgaatttatggcatgggtgctgaaagttcaggcggatctgtacttccacaacctgaaatttgatggcgcattcattatcaactggctggaacgtaatggctttaaatggagcgcggatggtctgccgaacacgtataataccattatctctcgtatgggccagtggtatatgattgatatctgcctgggctacaaaggtaaacgcaaaattcataccgtgatctatgatagcctgaaaaaactgccgtttccggtgaagaaaattgcgaaagatttcaaactgacggttctgaaaggcgatattgattatcacaaagaacgtccggttggttacaaaatcaccccggaagaatacgcatacatcaaaaacgatatccagatcatcgcagaagcgctgctgattcagtttaaacagggcctggatcgcatgaccgcgggcagtgatagcctgaaaggtttcaaagatatcatcacgaccaaaaaattcaaaaaagtgttcccgacgctgagcctgggtctggataaagaagttcgttatgcctaccgcggcggttttacctggctgaacgatcgtttcaaagaaaaagaaattggcgagggtatggtgtttgatgttaatagtctgtatccggcacagatgtacagccgcctgctgccgtatggcgaaccgatcgtgttcgagggtaaatatgtttgggatgaagattacccgctgcatattcagcacatccgttgtgaatttgaactgaaagaaggctatattccgaccattcagatcaaacgtagtcgcttctataagggtaacgaatacctgaaaagctctggcggtgaaatcgcggatctgtggctgagtaacgtggatctggaactgatgaaagaacactacgatctgtacaacgttgaatacatcagcggcctgaaatttaaagccacgaccggtctgttcaaagatttcatcgataaatggacctacatcaaaacgacctctgaaggcgcgattaaacagctggccaaactgatgctgaacagcctgtatggcaaattcgcctctaatccggatgtgaccggtaaagttccgtacctgaaagaaaatggcgcactgggttttcgcctgggcgaagaagaaacgaaagatccggtgtataccccgatgggtgttttcattacggcctgggcacgttacacgaccatcaccgcggcccaggcatgctatgatcgcattatctactgtgataccgattctattcatctgacgggcaccgaaatcccggatgtgattaaagatatcgttgatccgaaaaaactgggttattgggcccacgaaagtacgtttaaacgtgcaaaatacctgcgccagaaaacctacatccaggatatctacatgaaagaagtggatggcaaactggttgaaggttctccggatgattacaccgatatcaaattcagtgtgaaatgcgccggcatgacggataaaatcaaaaaagaagtgaccttcgaaaacttcaaagttggtttcagccgcaaaatgaaaccgaaaccggtgcaggttccgggcggtgtggttctggtggatgatacgtttaccattaaatctggcggtagtgcgtggagccatccgcagttcgaaaaaggcggtggctctggtggcggttctggcggtagtgcctggagccacccgcagtttgaaaaataataa

SEQ ID NO: 6 - protein, 608 aa, bacteriophage phi AR29
MKHMPRKMYSCAFETTTKVEDCRVWAYGYMNIEDHSEYKIGNSLDEFMAWVLKVQADLYFHNLKFDGAFIINWLERNGFKWSADGLPNTYNTIISRMGQWYMIDICLGYKGKRKIHTVIYDSLKKLPFPVKKIAKDFKLTVLKGDIDYHKERPVGYKITPEEYAYIKNDIQIIAEALLIQFKQGLDRMTAGSDSLKGFKDIITTKKFKKVFPTLSLGLDKEVRYAYRGGFTWLNDRFKEKEIGEGMVFDVNSLYPAQMYSRLLPYGEPIVFEGKYVWDEDYPLHIQHIRCEFELKEGYIPTIQIKRSRFYKGNEYLKSSGGEIADLWLSNVDLELMKEHYDLYNVEYISGLKFKATTGLFKDFIDKWTYIKTTSEGAIKQLAKLMLNSLYGKFASNPDVTGKVPYLKENGALGFRLGEEETKDPVYTPMGVFITAWARYTTITAAQACYDRIIYCDTDSIHLTGTEIPDVIKDIVDPKKLGYWAHESTFKRAKYLRQKTYIQDIYMKEVDGKLVEGSPDDYTDIKFSVKCAGMTDKIKKEVTFENFKVGFSRKMKPKPVQVPGGVVLVDDTFTIKSGGSAWSHPQFEKGGGSGGGSGGSAWSHPQFEK

SEQ ID NO: 7 - DNA, 1458 bp, Escherichia coli
atgatgaacgatggcaaacagcagagcaccttcctgtttcatgattatgaaaccttcggtacccatccggccctggatcgtccggcgcagtttgcggccattcgcaccgatagcgaattcaatgtgattggcgaaccggaagtgttttattgcaaaccggccgatgattatctgccgcagccgggtgcggtgctgattaccggtattaccccgcaggaagcgcgcgcgaaaggtgaaaacgaagcggcgtttgccgcgcgcattcatagcctgtttaccgtgccgaaaacctgcattctgggctataacaatgtgcgcttcgatgatgaagttacccgtaatatcttttatcgtaacttttatgatccgtatgcgtggagctggcagcatgataacagccgttgggatctgctggatgtgatgcgcgcgtgctatgcgctgcgcccggaaggcattaattggccggaaaacgatgatggcctgccgagctttcgtctggaacatctgaccaaagccaacggcattgaacatagcaatgcccatgatgcgatggccgatgtttatgcgaccattgcgatggcgaaactggttaaaacccgtcagccgcgcctgtttgattatctgtttacccaccgtaacaaacacaaactgatggcgctgattgatgttccgcagatgaaaccgctggtgcatgtgagcggcatgtttggcgcctggcgcggcaacaccagctgggtggccccgctggcctggcacccggaaaatcgtaacgccgtgattatggttgatctggccggtgatattagcccgctgctggaactggatagcgataccctgcgtgaacgcctgtataccgccaaaaccgatctgggcgataatgccgccgtgccggtgaaactggttcacattaacaaatgcccggtgctggcccaggcgaacaccctgcgcccggaagatgcggatcgtctgggtattaatcgccagcattgtctggataatctgaaaatcctgcgtgaaaacccgcaggtgcgtgaaaaagtggtggcgatcttcgcggaagcggaaccgttcaccccgagcgataacgtggatgcgcagctgtataacggcttctttagcgatgccgatcgcgcggcgatgaaaatcgttctggaaaccgaaccgcgcaatctgccggcgctggatattacctttgttgataaacgtattgaaaaactgctgtttaattatcgtgcgcgcaattttccgggtaccctggattatgccgaacagcagcgttggctggaacatcgtcgtcaggttttcaccccggaatttctgcagggttatgcggatgaactgcagatgctggttcagcagtatgccgatgataaagaaaaagtggcgctgctgaaagcgctgtggcagtatgcggaagaaatcgtttctggctctggtcaccatcatcatcaccactaa

SEQ ID NO: 8 - protein, 485 aa, Escherichia coli
MMNDGKQQSTFLFHDYETFGTHPALDRPAQFAAIRTDSEFNVIGEPEVFYCKPADDYLPQPGAVLITGITPQEARAKGENEAAFAARIHSLFTVPKTCILGYNNVRFDDEVTRNIFYRNFYDPYAWSWQHDNSRWDLLDVMRACYALRPEGINWPENDDGLPSFRLEHLTKANGIEHSNAHDAMADVYATIAMAKLVKTRQPRLFDYLFTHRNKHKLMALIDVPQMKPLVHVSGMFGAWRGNTSWVAPLAWHPENRNAVIMVDLAGDISPLLELDSDTLRERLYTAKTDLGDNAAVPVKLVHINKCPVLAQANTLRPEDADRLGINRQHCLDNLKILRENPQVREKVVAIFAEAEPFTPSDNVDAQLYNGFFSDADRAAMKIVLETEPRNLPALDITFVDKRIEKLLFNYRARNFPGTLDYAEQQRWLEHRRQVFTPEFLQGYADELQMLVQQYADDKEKVALLKALWQYAEEIVSGSGHHHHHH

SEQ ID NO: 9 - DNA, 804 bp, Escherichia coli
atgaaatttgttagcttcaatatcaacggcctgcgcgcgcgcccgcatcagctggaagcgattgtggaaaaacatcagccggatgttattggtctgcaggaaaccaaagttcacgatgatatgtttccgctggaagaagtggcgaaactgggctataacgtgttttatcatggccagaaaggtcattatggcgtggccctgctgaccaaagaaaccccgatcgcggttcgtcgtggttttccgggtgatgatgaagaagcgcagcgtcgtattattatggcggaaattccgagcctgctgggcaatgtgaccgttattaacggctattttccgcagggcgaaagccgtgatcatccgattaaatttccggccaaagcgcagttctatcagaacctgcagaactatctggaaaccgaactgaaacgtgataatccggtgctgatcatgggcgatatgaacattagcccgaccgatctggatattggcattggcgaagaaaaccgtaaacgctggctgcgtaccggtaaatgcagctttctgccggaagaacgtgaatggatggatcgcctgatgagctggggcctggtggatacctttcgtcatgcgaacccgcagaccgccgatcgctttagctggtttgattatcgcagcaaaggttttgatgataaccgtggcctgcgcattgatctgctgctggcgagccagccgctggcggaatgctgcgttgaaaccggtattgattatgaaattcgcagcatggaaaaaccgagcgatcacgccccggtgtgggcgacctttcgccgc

SEQ ID NO: 10 - protein, 268 aa, Escherichia coli
MKFVSFNINGLRARPHQLEAIVEKHQPDVIGLQETKVHDDMFPLEEVAKLGYNVFYHGQKGHYGVALLTKETPIAVRRGFPGDDEEAQRRIIMAEIPSLLGNVTVINGYFPQGESRDHPIKFPAKAQFYQNLQNYLETELKRDNPVLIMGDMNISPTDLDIGIGEENRKRWLRTGKCSFLPEEREWMDRLMSWGLVDTFRHANPQTADRFSWFDYRSKGFDDNRGLRIDLLLASQPLAECCVETGIDYEIRSMEKPSDHAPVWATFRR

SEQ ID NO: 11 - DNA, 2000 bp, Thermus thermophilus
atgcgtgatcgtgtccgctggcgtgttctgtccctgccgccgctggctcaatggcgtgaagttatggctgccctggaagtgggtccggaagcggccctggcatattggcaccgcggttttcgtcgcaaagaagatctggacccgccgctggccctgctgccgctgaaaggcctgcgcgaagcagctgcgctgctggaagaagccctgcgtcagggtaaacgtattcgcgttcatggcgattatgacgccgatggcctgaccggtaccgcaattctggtccgtggtctggcggcactgggtgccgatgtgcatccgtttattccgcaccgcctggaagaaggctacggtgtgctgatggaacgtgttccggaacacctggaagcgagcgacctgttcctgacggtggattgcggtatcaccaaccatgccgaactgcgtgaactgctggaaaatggcgttgaagtcattgtgaccgatcatcacaccccgggtaaaaccccgtctccgggcctggtggttcacccggcgctgacgccggatctgaaagaaaaaccgaccggcgctggtgtcgtgtttctgctgctgtgggcactgcacgaacgtctgggtctgccgccgccgctggaatatgccgacctggctgccgttggtaccattgccgatgttgccccgctgtggggttggaaccgtgcactggtgaaagaaggcctggcacgtattccggctagctcttgggttggtctgcgtctgctggccgaagcagtcggctacaccggtaaagcggttgaagtcgccttccgtattgcaccgcgcatcaacgccgcatcacgcctgggtgaagcagaaaaagctctgcgtctgctgctgacggatgacgctgcggaagctcaggcgctggttggcgaactgcaccgcctgaatgctcgtcgccagaccctggaagaagcgatgctgcgtaaactgctgccgcaagcggacccggaagccaaagcaatcgtgctgctggatccggaaggccatccgggtgttatgggcattgtcgcttcacgcatcctggaagcgacgctgcgtccggtctttctggtggcgcagggtaaaggtaccgtgcgcagcctggcaccgatttctgccgttgaagccctgcgtagcgccgaagacctgctgctgcgttatggcggtcacaaagaagccgcaggctttgctatggatgaagcgctgtttccggcattcaaagctcgcgttgaagcctacgctgcccgtttcccggacccggttcgtgaagtcgcactgctggatctgctgccggaaccgggtctgctgccgcaggtgtttcgtgaactggcgctgctggaaccgtatggcgaaggtaatccggaaccgctgtttctgctgtttggtgcaccggaagaagcacgtcgcctgggtgaaggtcgtcacctggcattccgcctgaaaggtgtgcgtgttctggcttggaaacagggtgatctggccctgccgccggaagttgaagtggcaggtctgctgtccgaaaacgcatggaatggccatctggcctatgaagtgcaagcagttgatctgcgtaaaccggaagcgctggaaggcggtattgccccgtttgcatatccgctgccgctgctggaagctctggcccgtgcccgcctgggcgaaggtgtttatgtcccggaagacaacccggaaggtctggattacgcacgcaaagctggcttccgtctgctgccgccggaagaagcgggtctgtggctgggtctgccgccgcgcccggtgctgggtcgtcgcgtggaagttgcactgggccgtgaagcacgtgctcgcctgagtgcaccgccggttctgcataccccggaagctcgcctgaaagcgctggtgcaccgtcgcctgctgtttgcctatgaacgtcgccatccgggtctgttctccgaagcgctgctggcctactgggaagtcaatcgtgttcaggaaccggcgggtagtcctaa

SEQ ID NO: 12 - protein, 666 aa, Thermus thermophilus
MRDRVRWRVLSLPPLAQWREVMAALEVGPEAALAYWHRGFRRKEDLDPPLALLPLKGLREAAALLEEALRQGKRIRVHGDYDADGLTGTAILVRGLAALGADVHPFIPHRLEEGYGVLMERVPEHLEASDLFLTVDCGITNHAELRELLENGVEVIVTDHHTPGKTPSPGLVVHPALTPDLKEKPTGAGVVFLLLWALHERLGLPPPLEYADLAAVGTIADVAPLWGWNRALVKEGLARIPASSWVGLRLLAEAVGYTGKAVEVAFRIAPRINAASRLGEAEKALRLLLTDDAAEAQALVGELHRLNARRQTLEEAMLRKLLPQADPEAKAIVLLDPEGHPGVMGIVASRILEATLRPVFLVAQGKGTVRSLAPISAVEALRSAEDLLLRYGGHKEAAGFAMDEALFPAFKARVEAYAARFPDPVREVALLDLLPEPGLLPQVFRELALLEPYGEGNPEPLFLLFGAPEEARRLGEGRHLAFRLKGVRVLAWKQGDLALPPEVEVAGLLSENAWNGHLAYEVQAVDLRKPEALEGGIAPFAYPLPLLEALARARLGEGVYVPEDNPEGLDYARKAGFRLLPPEEAGLWLGLPPRPVLGRRVEVALGREARARLSAPPVLHTPEARLKALVHRRLLFAYERRHPGLFSEALLAYWEVNRVQEPAGSP

SEQ ID NO: 13 - DNA, 681 bp, Bacteriophage lambda
atgacaccggacattatcctgcagcgtaccgggatcgatgtgagagctgtcgaacagggggatgatgcgtggcacaaattacggctcggcgtcatcaccgcttcagaagttcacaacgtgatagcaaaaccccgctccggaaagaagtggcctgacatgaaaatgtcctacttccacaccctgcttgctgaggtttgcaccggtgtggctccggaagttaacgctaaagcactggcctggggaaaacagtacgagaacgacgccagaaccctgtttgaattcacttccggcgtgaatgttactgaatccccgatcatctatcgcgacgaaagtatgcgtaccgcctgctctcccgatggtttatgcagtgacggcaacggccttgaactgaaatgcccgtttacctcccgggatttcatgaagttccggctcggtggtttcgaggccataaagtcagcttacatggcccaggtgcagtacagcatgtgggtgacgcgaaaaaatgcctggtactttgccaactatgacccgcgtatgaagcgtgaaggcctgcattatgtcgtgattgagcgggatgaaaagtacatggcgagttttgacgagatcgtgccggagttcatcgaaaaaatggacgaggcactggctgaaattggttttgtatttggggagcaatggcgataa

SEQ ID NO: 14 - protein, 226 aa, Bacteriophage lambda
MTPDIILQRTGIDVRAVEQGDDAWHKLRLGVITASEVHNVIAKPRSGKKWPDMKMSYFHTLLAEVCTGVAPEVNAKALAWGKQYENDARTLFEFTSGVNVTESPIIYRDESMRTACSPDGLCSDGNGLELKCPFTSRDFMKFRLGGFEAIKSAYMAQVQYSMWVTRKNAWYFANYDPRMKREGLHYVVIERDEKYMASFDEIVPEFIEKMDEALAEIGFVFGEQWR

SEQ ID NO: 15 - protein, 184 aa, Mycobacterium smegmatis
GLDNELSLVDGQDRTLTVQQWDTFLNGVFPLDRNRLTREWFHSGRAKYIVAGPGADEFEGTLELGYQIGFPWSLGVGINFSYTTPNILIDDGDITAPPFGLNSVITPNLFPGVSISADLGNGPGIQEVATFSVDVSGPAGGVAVSNAHGTVTGAAGGVLLRPFARLIASTGDSVTTYGEPWNMN

SEQ ID NO: 16 - protein, 184 aa, Mycobacterium smegmatis
GLDNELSLVDGQDRTLTVQQWDTFLNGVFPLDRNRLTREWFHSGRAKYIVAGPGADEFEGTLELGYQIGFPWSLGVGINFSYTTPNILIDDGDITGPPFGLESVITPNLFPGVSISADLGNGPGIQEVATFSVDVSGPAGGVAVSNAHGTVTGAAGGVLLRPFARLIASTGDSVTTYGEPWNMN

SEQ ID NO: 17 - protein, 183 aa, Mycobacterium smegmatis
VDNQLSVVDGQGRTLTVQQAETFLNGVFPLDRNRLTREWFHSGRATYHVAGPGADEFEGTLELGYQVGFPWSLGVGINFSYTTPNILIDGGDITQPPFGLDTIITPNLFPGVSISADLGNGPGIQEVATFSVDVKGAKGAVAVSNAHGTVTGAAGGVLLRPFARLIASTGDSVTTYGEPWNMN

SEQ ID NO: 18 - DNA, 70 bp, Artificial sequence
  Sequence used in the examples
tttttttttttttttttttttttttttttttttttttttttttttttttttttttttttttttttttttt

SEQ ID NO: 19 - DNA, 70 bp, Artificial Sequence
  Sequence used in the examples
aaaaaaaaaaaaaaaaaaaaaaaaaaaaaaaaaaaaaaaaaaaaaaaaaaaaaaaaaaaaaaaaaaaaaa

SEQ ID NO: 20 - DNA, 70 bp, Artificial Sequence
  Sequence used in the examples
cccccccccccccccccccccccccccccccccccccccccccccccccccccccccccccccccccccc

SEQ ID NO: 21 - DNA, 70 bp, Artificial Sequence
  Sequence used in the examples
tgtgttctatgtcttattcttacttcgttattcttgtctctattctgtttatgtttcttgtttgttagca

SEQ ID NO: 22 - DNA, 93 bp, Artificial Sequence
  Sequence used in the examples
ttttttttttttttttttttttttttttttttttttttttttttttttttttttttttttttttttttttggctacgacctgcatgagaatgc

SEQ ID NO: 23 - DNA, 79 bp, Artificial Sequence
  Sequence used in the examples
ctcacctatccttccactcaccccccaaaaaaccccccaaaaaaccccccaaaaaagcattctcatgcaggtcgtagcc

SEQ ID NO: 24 - DNA, 100 bp, Artificial Sequence
  Sequence used in the examples
aacccccaaaaacccccaaaaacccccaaaaacccccaaaaacccccaaaaacccccaaaaacccccaaaaacccccatagagacaagaataacgaagta

SEQ ID NO: 25 - DNA, 23 bp, Artificial Sequence
  Sequence used in the examples
tacttcgttattcttgtctctat

SEQ ID NO: 26 - DNA, 65 bp, Artificial Sequence
  Sequence used in the examples
cccccccccccccccaccccccccccccccccccctattctgtttatgtttcttgtttgttagcc

SEQ ID NO: 27 - DNA, 31 bp, Artificial Sequence
  Sequence used in the examples
ggctaacaaacaagaaacataaacagaatag

SEQ ID NO: 28 - DNA, 65 bp, Artificial sequence; identical to SEQ ID NO: 26
  Sequence used in the examples

SEQ ID NO: 29 - DNA, 81 bp, Artificial Sequence
  Sequence used in the examples
  misc_feature (51)..(54): n = abasic nucleotide
ttttttttttttttttttttttttttttttttttttttttttttttttttnnnnggttgtttctgttggtgctgatattgc

SEQ ID NO: 30 - DNA, 27 bp, Artificial Sequence
  Sequence used in examples
gttagaccaaaccatgaaaccaacata

SEQ ID NO: 31 - DNA, 24 bp, Artificial Sequence
  Sequence used in examples
gaccgcctccaaacaatttagaca

SEQ ID NO: 32 - DNA, 24 bp, Artificial Sequence
  Sequence used in the examples
ggcaatctctttctgattgtccag

SEQ ID NO: 33 - DNA, 885 bp, Artificial sequence
  sequence for one subunit of alpha-HL-Q
atggcagattctgatattaatattaaaaccggtactacagatattggaagcaatactacagtaaaaacaggtgatttagtcacttatgataaagaaaatggcatgcacaaaaaagtattttatagttttatcgatgataaaaatcacaataaaaaactgctagttattagaacaaaaggtaccattgctggtcaatatagagtttatagcgaagaaggtgctaacaaaagtggtttagcctggccttcagcctttaaggtacagttgcaactacctgataatgaagtagctcaaatatctgattactatccaagaaattcgattgatacaaaagagtatatgagtactttaacttatggattcaacggtaatgttactggtgatgatacaggaaaaattggcggccttattggtgcacaagtttcgattggtcatacactgaaatatgttcaacctgatttcaaaacaattttagagagcccaactgataaaaaagtaggctggaaagtgatatttaacaatatggtgaatcaaaattggggaccatacgatcgagattcttggaacccggtatatggcaatcaacttttcatgaaaactagaaatggttctatgaaagcagcagataacttccttgatcctaacaaagcaagttctctattatcttcagggttttcaccagacttcgctacagttattactatggatagaaaagcatccaaacaacaaacaaatatagatgtaatatacgaacgagttcgtgatgattaccaattgcattggacttcaacaaattggaaaggtaccaatactaaagataaatggacagatcgttcttcagaaagatataaaatcgattgggaaaaagaagaaatgacaaattaa

SEQ ID NO: 34 - protein, 293 aa, Artificial Sequence
  protein sequence for one subunit of alpha-HL-Q
ADSDINIKTGTTDIGSNTTVKTGDLVTYDKENGMHKKVFYSFIDDKNHNKKLLVIRTKGTIAGQYRVYSEEGANKSGLAWPSAFKVQLQLPDNEVAQISDYYPRNSIDTKEYMSTLTYGFNGNVTGDDTGKIGGLIGAQVSIGHTLKYVQPDFKTILESPTDKKVGWKVIFNNMVNQNWGPYDRDSWNPVYGNQLFMKTRNGSMKAADNFLDPNKASSLLSSGFSPDFATVITMDRKASKQQTNIDVIYERVRDDYQLHWTSTNWKGTNTKDKWTDRSSERYKIDWEKEEMTN

SEQ ID NO: 35 - DNA, 957 bp, Artificial Sequence
  polynucleotide sequence of one subunit of alpha-HL-E287C-QC-D5FLAG
atggcagattctgatattaatattaaaaccggtactacagatattggaagcaatactacagtaaaaacaggtgatttagtcacttatgataaagaaaatggcatgcacaaaaaagtattttatagttttatcgatgataaaaatcacaataaaaaactgctagttattagaacaaaaggtaccattgctggtcaatatagagtttatagcgaagaaggtgctaacaaaagtggtttagcctggccttcagcctttaaggtacagttgcaactacctgataatgaagtagctcaaatatctgattactatccaagaaattcgattgatacaaaagagtatatgagtactttaacttatggattcaacggtaatgttactggtgatgatacaggaaaaattggcggctgtattggtgcacaagtttcgattggtcatacactgaaatatgttcaacctgatttcaaaacaattttagagagcccaactgataaaaaagtaggctggaaagtgatatttaacaatatggtgaatcaaaattggggaccatacgatcgagattcttggaacccggtatatggcaatcaacttttcatgaaaactagaaatggttctatgaaagcagcagataacttccttgatcctaacaaagcaagttctctattatcttcagggttttcaccagacttcgctacagttattactatggatagaaaagcatccaaacaacaaacaaatatagatgtaatatacgaacgagttcgtgatgattaccaattgcattggacttcaacaaattggaaaggtaccaatactaaagataaatggacagatcgttcttcagaaagatataaaatcgattggtgcaaagaagaaatgacaaatgatgatgatgatgatagcggcagcggtgattataaagatgatgatgataaagcgcaccatcatcatcaccactaa

SEQ ID NO: 36 - protein, 317 aa, Artificial Sequence
  amino acid sequence of one subunit of alpha-HL-E287C-QC-D5FLAG
ADSDINIKTGTTDIGSNTTVKTGDLVTYDKENGMHKKVFYSFIDDKNHNKKLLVIRTKGTIAGQYRVYSEEGANKSGLAWPSAFKVQLQLPDNEVAQISDYYPRNSIDTKEYMSTLTYGFNGNVTGDDTGKIGGCIGAQVSIGHTLKYVQPDFKTILESPTDKKVGWKVIFNNMVNQNWGPYDRDSWNPVYGNQLFMKTRNGSMKAADNFLDPNKASSLLSSGFSPDFATVITMDRKASKQQTNIDVIYERVRDDYQLHWTSTNWKGTNTKDKWTDRSSERYKIDWCKEEMTNDDDDDSGSGDYKDDDDKAHHHHHH

SEQ ID NO: 37 - DNA, 885 bp, Artificial sequence
  polynucleotide sequence of one subunit of alpha-hemolysin-E111N/K147N
atggcagattctgatattaatattaaaaccggtactacagatattggaagcaatactacagtaaaaacaggtgatttagtcacttatgataaagaaaatggcatgcacaaaaaagtattttatagttttatcgatgataaaaatcacaataaaaaactgctagttattagaacaaaaggtaccattgctggtcaatatagagtttatagcgaagaaggtgctaacaaaagtggtttagcctggccttcagcctttaaggtacagttgcaactacctgataatgaagtagctcaaatatctgattactatccaagaaattcgattgatacaaaaaactatatgagtactttaacttatggattcaacggtaatgttactggtgatgatacaggaaaaattggcggccttattggtgcaaatgtttcgattggtcatacactgaactatgttcaacctgatttcaaaacaattttagagagcccaactgataaaaaagtaggctggaaagtgatatttaacaatatggtgaatcaaaattggggaccatacgatcgagattcttggaacccggtatatggcaatcaacttttcatgaaaactagaaatggttctatgaaagcagcagataacttccttgatcctaacaaagcaagttctctattatcttcagggttttcaccagacttcgctacagttattactatggatagaaaagcatccaaacaacaaacaaatatagatgtaatatacgaacgagttcgtgatgattaccaattgcattggacttcaacaaattggaaaggtaccaatactaaagataaatggacagatcgttcttcagaaagatataaaatcgattgggaaaaagaagaaatgacaaattaa

SEQ ID NO: 38 - protein, 293 aa, artificial sequence
  amino acid sequence of one subunit of alpha-hemolysin-E111N/K147N
ADSDINIKTGTTDIGSNTTVKTGDLVTYDKENGMHKKVFYSFIDDKNHNKKLLVIRTKGTIAGQYRVYSEEGANKSGLAWPSAFKVQLQLPDNEVAQISDYYPRNSIDTKNYMSTLTYGFNGNVTGDDTGKIGGLIGANVSIGHTLNYVQPDFKTILESPTDKKVGWKVIFNNMVNQNWGPYDRDSWNPVYGNQLFMKTRNGSMKAADNFLDPNKASSLLSSGFSPDFATVITMDRKASKQQTNIDVIYERVRDDYQLHWTSTNWKGTNTKDKWTDRSSERYKIDWEKEEMTN

SEQ ID NO: 39 - DNA, 518 bp, Artificial Sequence
  Sequence used in the examples
ttttttttttttttttttttttttttttttttttttttttttttttttttggttgtttctgttggtgctgatattgcgctccactaaagggccgattgacccggtggtaccttggttgtttctgttggtgctgatattgcttttgatgccgaccctaaattttttgcctgtttggttcgctttgagtcttcttcggttccgactaccctcccgactgcctatgatgtttatcctttggatggtcgccatgatggtggttattataccgtcaaggactgtgtgactattgacgtccttccccgtacgccgggcaataatgtttatgttggtttcatggtttggtctaactttaccgctactaaatgccgcggattggtttcgctgaatcaggttattaaagagattatttgtctccagccacttaagtgaggtgatttatgtttggtgctattgctggcggtattgcttctgctcttgctggtggcgccatgtctaaattgtttggaggcggtcgagct

SEQ ID NO: 40 - DNA, 530 bp, Artificial Sequence
  Sequence used in the example
ttttttttttttttttttttttttttttttttttttttttttttttttttggttgtttctgttggtgctgatattgcgctccactaaagggccgattgacgctccactaaagggccgattgacccggttgtttctgttggtgctgatattgcttttgatgccgaccctaaattttttgcctgtttggttcgctttgagtcttcttcggttccgactaccctcccgactgcctatgatgtttatcctttggatggtcgccatgatggtggttattataccgtcaaggactgtgtgactattgacgtccttccccgtacgccgggcaataatgtttatgttggtttcatggtttggtctaactttaccgctactaaatgccgcggattggtttcgctgaatcaggttattaaagagattatttgtctccagccacttaagtgaggtgatttatgtttggtgctattgctggcggtattgcttctgctcttgctggtggcgccatgtctaaattgtttggaggcggtcgagct

SEQ ID NO: 41 - DNA, 57 bp, Artificial Sequence
  Sequence used in the examples
agcgactaacaaacacaatctgatggctttttttttttttttttttttttttttttt